European Patent Specification EP 3 497 452 B1, published March 5, 2025. Title: DIAGNOSIS, PREVENTION, AND/OR TREATMENT OF AUTOIMMUNE DISEASES. Applicant: IMMUNOWORK, LLC. The sequence listing filed with the application follows.

SEQUENCE LISTING (17 sequences)

SEQ ID NO: 1 - protein, 658 aa, Artificial
  Synthetic
MLLSPSLLLLLLLGAPRGCAEGVAAALTPERLLEWQDKGIFVIQSESLKKCIQAGKSVLTLENCKQANKHMLWKWVSNHGLFNIGGSGCLGLNFSAPEQPLSLYECDSTLVSLRWRCNRKMITGPLQYSVQVAHDNTVVASRKYIHKWISYGSGGGDICEYLHKDLHTIKGNTHGMPCMFPFQYNHQWHHECTREGREDDLLWCATTSRYERDEKWGFCPDPTSAEVGCDTIWEKDLNSHICYQFNLLSSLSWSEAHSSCQMQGGTLLSITDETEENFIREHMSSKTVEVWMGLNQLDEHAGWQWSDGTPLNYLNWSPEVNFEPFVEDHCGTFSSFMPSAWRSRDCESTLPYICKKYLNHIDHEIVEKDAWKYYATHCEPGWNPYNRNCYKLQKEEKTWHEALRSCQADNSALIDITSLAEVEFLVTLLGDENASETWIGLSSNKIPVSFEWSNDSSVIFTNWHTLEPHIFPNRSQLCVSAEQSEGHWKVKNCEERLFYICKKAGHVLSDAESGCQEGWERHGGFCYKIDTVLRSFDQASSGYYCPPALVTITNRFEQAFITSLISSVVKMKDSYFWIALQDQNDTGEYTWKPVGQKPEPVQYTHWNTHQPRYSGGCVAMRGRHPLGRWEVKHCRHFKAMSLCKQPVENQEKAEYEER

SEQ ID NO: 2 - protein, 364 aa, Artificial
  Synthetic
MLLSPSLLLLLLLGAPRGCAEGVAAALTPERLLEWQDKGIFVIQSESLKKCIQAGKSVLTLENCKQANKHMLWKWVSNHGLFNIGGSGCLGLNFSAPEQPLSLYECDSTLVSLRWRCNRKMITGPLQYSVQVAHDNTVVASRKYIHKWISYGSGGGDICEYLHKDLHTIKGNTHGMPCMFPFQYNHQWHHECTREGREDDLLWCATTSRYERDEKWGFCPDPTSAEVGCDTIWEKDLNSHICYQFNLLSSLSWSEAHSSCQMQGGTLLSITDETEENFIREHMSSKTVEVWMGLNQLDEHAGWQWSDGTPLNYLNWSPEVNFEPFVEDHCGTFSSFMPSAWRSRDCESTLPYICKKYLNHIDHE

SEQ ID NO: 3 - protein, 294 aa, Artificial
  Synthetic
IVEKDAWKYYATHCEPGWNPYNRNCYKLQKEEKTWHEALRSCQADNSALIDITSLAEVEFLVTLLGDENASETWIGLSSNKIPVSFEWSNDSSVIFTNWHTLEPHIFPNRSQLCVSAEQSEGHWKVKNCEERLFYICKKAGHVLSDAESGCQEGWERHGGFCYKIDTVLRSFDQASSGYYCPPALVTITNRFEQAFITSLISSVVKMKDSYFWIALQDQNDTGEYTWKPVGQKPEPVQYTHWNTHQPRYSGGCVAMRGRHPLGRWEVKHCRHFKAMSLCKQPVENQEKAEYEER

SEQ ID NO: 4 - protein, 805 aa, Artificial
  Synthetic
MLLSPSLLLLLLLGAPRGCAEGVAAALTPERLLEWQDKGIFVIQSESLKKCIQAGKSVLTLENCKQANKHMLWKWVSNHGLFNIGGSGCLGLNFSAPEQPLSLYECDSTLVSLRWRCNRKMITGPLQYSVQVAHDNTVVASRKYIHKWISYGSGGGDICEYLHKDLHTIKGNTHGMPCMFPFQYNHQWHHECTREGREDDLLWCATTSRYERDEKWGFCPDPTSAEVGCDTIWEKDLNSHICYQFNLLSSLSWSEAHSSCQMQGGTLLSITDETEENFIREHMSSKTVEVWMGLNQLDEHAGWQWSDGTPLNYLNWSPEVNFEPFVEDHCGTFSSFMPSAWRSRDCESTLPYICKKYLNHIDHEIVEKDAWKYYATHCEPGWNPYNRNCYKLQKEEKTWHEALRSCQADNSALIDITSLAEVEFLVTLLGDENASETWIGLSSNKIPVSFEWSNDSSVIFTNWHTLEPHIFPNRSQLCVSAEQSEGHWKVKNCEERLFYICKKAGHVLSDAESGCQEGWERHGGFCYKIDTVLRSFDQASSGYYCPPALVTITNRFEQAFITSLISSVVKMKDSYFWIALQDQNDTGEYTWKPVGQKPEPVQYTHWNTHQPRYSGGCVAMRGRHPLGRWEVKHCRHFKAMSLCKQPVENQEKAEYEERWPFHPCYLDWESEPGLASCFKVFHSEKVLMKRTWREAEAFCEEFGAHLASFAHIEEENFVNELLHSKFNWTEERQFWIGFNKRNPLNAGSWEWSDRTPVVSSFLDNTYFGEDARNCAVYKANKTLLPLHCGSKREWICKIPRDVKPK

SEQ ID NO: 5 - protein, 367 aa, Artificial
  Synthetic
MLLSPSLLLLLLLGAPRGCAEGVAAALTPERLLEWQDKGIFVIQSESLKKCIQAGKSVLTLENCKQANKHMLWKWVSNHGLFNIGGSGCLGLNFSAPEQPLSLYECDSTLVSLRWRCNRKMITGPLQYSVQVAHDNTVVASRKYIHKWISYGSGGGDICEYLHKDLHTIKGNTHGMPCMFPFQYNHQWHHECTREGREDDLLWCATTSRYERDEKWGFCPDPTSAEVGCDTIWEKDLNSHICYQFNLLSSLSWSEAHSSCQMQGGTLLSITDETEENFIREHMSSKTVEVWMGLNQLDEHAGWQWSDGTPLNYLNWSPEVNFEPFVEDHCGTFSSFMPSAWRSRDCESTLPYICKKYLNHIDHEIVE

SEQ ID NO: 6 - protein, 438 aa, Artificial
  Synthetic
KDAWKYYATHCEPGWNPYNRNCYKLQKEEKTWHEALRSCQADNSALIDITSLAEVEFLVTLLGDENASETWIGLSSNKIPVSFEWSNDSSVIFTNWHTLEPHIFPNRSQLCVSAEQSEGHWKVKNCEERLFYICKKAGHVLSDAESGCQEGWERHGGFCYKIDTVLRSFDQASSGYYCPPALVTITNRFEQAFITSLISSVVKMKDSYFWIALQDQNDTGEYTWKPVGQKPEPVQYTHWNTHQPRYSGGCVAMRGRHPLGRWEVKHCRHFKAMSLCKQPVENQEKAEYEERWPFHPCYLDWESEPGLASCFKVFHSEKVLMKRTWREAEAFCEEFGAHLASFAHIEEENFVNELLHSKFNWTEERQFWIGFNKRNPLNAGSWEWSDRTPVVSSFLDNTYFGEDARNCAVYKANKTLLPLHCGSKREWICKIPRDVKPK

SEQ ID NO: 7 - protein, 169 aa, Artificial
  Synthetic
MLLSPSLLLLLLLGAPRGCAEGVAAALTPERLLEWQDKGIFVIQSESLKKCIQAGKSVLTLENCKQANKHMLWKWVSNHGLFNIGGSGCLGLNFSAPEQPLSLYECDSTLVSLRWRCNRKMITGPLQYSVQVAHDNTVVASRKYIHKWISYGSGGGDICEYLHKDLHTI

SEQ ID NO: 8 - protein, 228 aa, Artificial
  Synthetic
MLLSPSLLLLLLLGAPRGCAEGVAAALTPERLLEWQDKGIFVIQSESLKKCIQAGKSVLTLENCKQANKHMLWKWVSNHGLFNIGGSGCLGLNFSAPEQPLSLYECDSTLVSLRWRCNRKMITGPLQYSVQVAHDNTVVASRKYIHKWISYGSGGGDICEYLHKDLHTIKGNTHGMPCMFPFQYNHQWHHECTREGREDDLLWCATTSRYERDEKWGFCPDPTSAEVG

SEQ ID NO: 9 - protein, 367 aa, Artificial; identical to SEQ ID NO: 5
  Synthetic

SEQ ID NO: 10 - protein, 510 aa, Artificial
  Synthetic
MLLSPSLLLLLLLGAPRGCAEGVAAALTPERLLEWQDKGIFVIQSESLKKCIQAGKSVLTLENCKQANKHMLWKWVSNHGLFNIGGSGCLGLNFSAPEQPLSLYECDSTLVSLRWRCNRKMITGPLQYSVQVAHDNTVVASRKYIHKWISYGSGGGDICEYLHKDLHTIKGNTHGMPCMFPFQYNHQWHHECTREGREDDLLWCATTSRYERDEKWGFCPDPTSAEVGCDTIWEKDLNSHICYQFNLLSSLSWSEAHSSCQMQGGTLLSITDETEENFIREHMSSKTVEVWMGLNQLDEHAGWQWSDGTPLNYLNWSPEVNFEPFVEDHCGTFSSFMPSAWRSRDCESTLPYICKKYLNHIDHEIVEKDAWKYYATHCEPGWNPYNRNCYKLQKEEKTWHEALRSCQADNSALIDITSLAEVEFLVTLLGDENASETWIGLSSNKIPVSFEWSNDSSVIFTNWHTLEPHIFPNRSQLCVSAEQSEGHWKVKNCEERLFYICKKAGHVLSD

SEQ ID NO: 11 - protein, 651 aa, Artificial
  Synthetic
MLLSPSLLLLLLLGAPRGCAEGVAAALTPERLLEWQDKGIFVIQSESLKKCIQAGKSVLTLENCKQANKHMLWKWVSNHGLFNIGGSGCLGLNFSAPEQPLSLYECDSTLVSLRWRCNRKMITGPLQYSVQVAHDNTVVASRKYIHKWISYGSGGGDICEYLHKDLHTIKGNTHGMPCMFPFQYNHQWHHECTREGREDDLLWCATTSRYERDEKWGFCPDPTSAEVGCDTIWEKDLNSHICYQFNLLSSLSWSEAHSSCQMQGGTLLSITDETEENFIREHMSSKTVEVWMGLNQLDEHAGWQWSDGTPLNYLNWSPEVNFEPFVEDHCGTFSSFMPSAWRSRDCESTLPYICKKYLNHIDHEIVEKDAWKYYATHCEPGWNPYNRNCYKLQKEEKTWHEALRSCQADNSALIDITSLAEVEFLVTLLGDENASETWIGLSSNKIPVSFEWSNDSSVIFTNWHTLEPHIFPNRSQLCVSAEQSEGHWKVKNCEERLFYICKKAGHVLSDAESGCQEGWERHGGFCYKIDTVLRSFDQASSGYYCPPALVTITNRFEQAFITSLISSVVKMKDSYFWIALQDQNDTGEYTWKPVGQKPEPVQYTHWNTHQPRYSGGCVAMRGRHPLGRWEVKHCRHFKAMSLCKQPVENQE

SEQ ID NO: 12 - protein, 805 aa, Artificial; identical to SEQ ID NO: 4
  Synthetic

SEQ ID NO: 13 - protein, 139 aa, Artificial
  Synthetic
CDTIWEKDLNSHICYQFNLLSSLSWSEAHSSCQMQGGTLLSITDETEENFIREHMSSKTVEVWMGLNQLDEHAGWQWSDGTPLNYLNWSPEVNFEPFVEDHCGTFSSFMPSAWRSRDCESTLPYICKKYLNHIDHEIVE

SEQ ID NO: 14 - protein, 1462 aa, Artificial
  Synthetic
MLLSPSLLLLLLLGAPRGCAEGVAAALTPERLLEWQDKGIFVIQSESLKKCIQAGKSVLTLENCKQANKHMLWKWVSNHGLFNIGGSGCLGLNFSAPEQPLSLYECDSTLVSLRWRCNRKMITGPLQYSVQVAHDNTVVASRKYIHKWISYGSGGGDICEYLHKDLHTIKGNTHGMPCMFPFQYNHQWHHECTREGREDDLLWCATTSRYERDEKWGFCPDPTSAEVGCDTIWEKDLNSHICYQFNLLSSLSWSEAHSSQMQGGTLLSITDETEENFIREHMSSKTVEVWMGLNQLDEHAGWQWSDGTPLNYLNWSPEVNFEPFVEDHCGTFSSFMPSAWRSRDCESTLPYICKKYLNHIDHEIVEKDAWKYYATHCEPGWNPYNRNCYKLQKEEKTWHEALRSCQADNSALIDITSLAEVEFLVTLLGDENASETWIGLSSNKIPVSFEWSNDSSVIFTNWHTLEPHIFPNRSQLCVSAEQSEGHWKVKNCEERLFYICKKAGHVLSDAESGCQEGWERHGGFCYKIDTVLRSFDQASSGYYCPPALVTITNRFEQAFITSLISSVVKMKDSYFWIALQDQNDTGEYTWKPVGQKPEPVQYTHWNTHQPRYSGGCVAMRGRHPLGRWEVKHCRHFKAMSLCKQPVENQEKAEYEERWPFHPCYLDWESEPGLASCFKVFHSEKVLMKRTWREAEAFCEEFGAHLASFAHIEEENFVNELLHSKFNWTEERQFWIGFNKRNPLNAGSWEWSDRTPVVSSFLDNTYFGEDARNCAVYKANKTLLPLHCGSKREWICKIPRDVKPKIPFWYQYDVPWLFYQDAEYLFHTFASEWLNFEFVCSWLHSDLLTIHSAHEQEFIHSKIKALSKYGASWWIGLQEERANDEFRWRDGTPVIYQNWDTGRERTVNNQSQRCGFISSITGLWGSEECSVSMPSICKRKKVWLIEKKKDTPKQHGTCPKGWLYFNYKCLLLNIPKDPSSWKNWTHAQHFCAEEGGTLVAIESEVEQAFITMNLFGQTTSVWIGLQNDDYETWLNGKPVVYSNWSPFDIINIPSHNTTEVQKHIPLCALLSSNPNFHFTGKWYFEDCGKEGYGFVCEKMQDTSGHGVNTSDMYPMPNTLEYGNRTYKIINANMTWYAAIKTCLMHKAQLVSITDQYHQSFLTVVLNRLGYAHWIGLFTTDNGLNFDWSDGTKSSFTFWKDEESSLLGDCVFADSNGRWHSTACESFLQGAICHVPPETRQSEHPELCSETSIPWIKFKSNCYSFSTVLDSMSFEAAHEFCKKEGSNLLTIKDEAENAFLLEELFAFGSSVQMVWLNAQFDGNNETIKWFDGTPTDQSNWGIRKPDTDYFKPHHCVALRIPEGLWQLSPCQEKKGFICKMEADIHTAEALPEKGPSHSIIPLAVVLTLIVIVAICTLSFCIYKHNGGFFRRLAGFRNPYYPATNFSTVYLEENILISDLEKSDQ

SEQ ID NO: 15 - protein, 272 aa, Artificial
  Synthetic
MDSYLLMWGLLTFIMVPGCQAELCDDDPPEIPHATFKAMAYKEGTMLNCECKRGFRRIKSGSLYMLCTGNSSHSSWDNQCQCTSSATRNTTKQVTPQPEEQKERKTTEMQSPMQPVDQASLPGHCREPPPWENEATERIYHFVVGQMVYYQCVQGYRALHRGPAESVCKMTHGKTRWTQPQLICTGEMETSQFPGEEKPQASPEGRPESETSCLVTTTDFQIQTEMAATMETSIFTTEYQVAVAGCVFLLISVLLLSGLTWQRRQRKSRRTI

SEQ ID NO: 16 - protein, 336 aa, Artificial
  Synthetic
EWIKFAAACREGEDNSKRNPIAKIHSDCAANQQVTYRISGVGIDQPPYGIFVINQKTGEINITSIVDREVTPFFIIYCRALNSMGQDLERPLELRVRVLDINDNPPVFSMATFAGQIEENSNANTLVMILNATDADEPNNLNSKIAFKIIRQEPSDSPMFIINRNTGEIRTMNNFLDREQYGQYALAVRGSDRDGGADGMSAECECNIKILDVNDNIPYMEQSSYTIEIQENTLNSNLLEIRVIDLDEEFSANWMAVIFFISGNEGNWFEIEMNERTNVGILKVVKPLDYEAMQSLQLSIGVRNKAEFHHSIMSQYKLKASAISVTVLNVIEGPVF

SEQ ID NO: 17 - protein, 450 aa, Artificial
  Synthetic
EWVKFAKPCREGEDNSKRNPIAKITSDYQATQKITYRISGVGIDQPPFGIFVVDKNTGDINITAIVDREETPSFLITCRALNAQGLDVEKPLILTVKILDINDNPPVFSQQIFMGEIEENSASNSLVMILNATDADEPNHLNSKIAFKIVSQEPAGTPMFLLSRNTGEVRTLTNSLDREQASSYRLVVSGADKDGEGLSTQCECNIKVKDVNDNFPMFRDSQYSARIEENILSSELLRFQVTDLDEEYTDNWLAVYFFTSGNEGNWFEIQTDPRTNEGILKVVKALDYEQLQSVKLSIAVKNKAEFHQSVISRYRVQSTPVTIQVINVREGIAFRPASKTFTVQKGISSKKLVDYILGTYQAIDEDTNKAASNVKYVMGRNDGGYLMIDSKTAEIKFVKNMNRDSTFIVNKTITAEVLAIDEYTGKTSTGTVYVRVPDFNDNCPTAVLEK